European Patent Application EP 4 685 153 A1, published January 28, 2026. Title: BROAD-SPECTRUM VIRAL MEMBRANE FUSION INHIBITOR, AND PREPARATION METHOD THEREFOR AND USE THEREOF. Applicant: HENAN GENUINE BIOTECH CO., LTD. Application WO PCT/CN2023/082491, filed March 20, 2023. The sequence listing filed with the application follows.

SEQUENCE LISTING (29 sequences)

SEQ ID NO: 1 - protein, 36 aa, synthetic construct
  SITE 36: note = The C-terminus is modified by an amino group
  SITE 1: note = The N-terminus is modified by an acetyl group
YTSLIHSLIEESQNQQEKNEQELLELDKWASLWNWF

SEQ ID NO: 2 - protein, 34 aa, synthetic construct
  SITE 1: note = The N-terminus is modified by an acetyl group
  SITE 34: note = The C-terminus is modified by an amino group
WMEWDREINNYTSLIHSLIEESQNQQEKNEQELL

SEQ ID NO: 3 - protein, 39 aa, synthetic construct
  SITE 1: note = The N-terminus is modified by an acetyl group
  SITE 39: note = The C-terminus is modified by an amino group
WQEWEQKITALLEQAQIQQEKNEYELQKLDKWASLWEWF

SEQ ID NO: 4 - protein, 38 aa, synthetic construct
  SITE 1: note = The N-terminus is modified by an acetyl group
  SITE 38: note = The C-terminus is modified by an amino group
TTWEAWDRAIAEYAARIEALIRAAQEQQEKNEAALREL

SEQ ID NO: 5 - protein, 36 aa, synthetic construct
  SITE 1: note = The N-terminus is modified by an acetyl group
  SITE 36: note = The C-terminus is modified by an amino group
SWETWEREIENYTRQIYRILEESQEQQDRNERDLLE

SEQ ID NO: 6 - protein, 34 aa, synthetic construct
  SITE 1: note = The N-terminus is modified by an acetyl group
  SITE 34: note = The C-terminus is modified by an amino group
WEEWDREINNYTKLIHELIEESQNQQEKNEQELL

SEQ ID NO: 7 - protein, 38 aa, synthetic construct
  SITE 1: note = The N-terminus is modified by an acetyl group
  SITE 38: note = The C-terminus is modified by an amino group
  SITE 38: note = The C-terminal is modified by a cholesterol molecule
WMEWDREINNYTSLIHSLIEESQNQQEKNEQELLGSGC

SEQ ID NO: 8 - protein, 24 aa, synthetic construct
  SITE 1: note = The N-terminus is modified by an acetyl group
  SITE 24: note = The C-terminus is modified by an amino group
  SITE 24: note = The C-terminus is modified by a palmitic acid molecule
EMTWEEWEKKIEEYTKKIEEILKK

SEQ ID NO: 9 - protein, 28 aa, synthetic construct
  SITE 1: note = The N-terminus is modified by an acetyl group
  SITE 28: note = The C-terminus is modified by an amino group
  SITE 28: note = The C-terminal is modified by a cholesterol molecule
YEQKIEELLKKAEEQQKKNEEELKKLEK

SEQ ID NO: 10 - protein, 40 aa, synthetic construct
  SITE 1: note = The N-terminus is modified by an acetyl group
  SITE 40: note = The C-terminus is modified by an amino group
  SITE 40: note = The C-terminal is modified by a cholesterol molecule
WMEWDREINNYTSLIHSLIEESQNQQEKNEQELLGSGSGK

SEQ ID NO: 11 - protein, 40 aa, synthetic construct
  SITE 1: note = The N-terminus is modified by an acetyl group
  SITE 40: note = The C-terminus is modified by an amino group
  SITE 40: note = The C-terminal is modified by a cholesterol molecule
WMEWDREINNYTSLIHSLIEESQNQQEKNEQELLEAAAKK

SEQ ID NO: 12 - protein, 38 aa, synthetic construct
  SITE 1: note = The N-terminus is modified by an acetyl group
  SITE 38: note = The C-terminus is modified by an amino group
  SITE 38: note = The C-terminal is modified by a cholesterol molecule
EMTWEEWEKKIEELEKKIEELLKKAEEQQKKNEAAAKK

SEQ ID NO: 13 - protein, 38 aa, synthetic construct
  SITE 1: note = The N-terminus is modified by an acetyl group
  SITE 38: note = The C-terminus is modified by an amino group
  SITE 38: note = The C-terminal is modified by a cholesterol molecule
TWEEWEKKIEELEKKIEELLKKAEEQQKKNEQEAAAKK

SEQ ID NO: 14 - protein, 36 aa, synthetic construct
  SITE 1: note = The N-terminus is modified by an acetyl group
  SITE 36: note = The C-terminus is modified by an amino group
  SITE 36: note = The C-terminal is modified by a cholesterol molecule
TWEEWEKKIEELEKKIEELLKKAEEQQKKNEAAAKK

SEQ ID NO: 15 - protein, 38 aa, synthetic construct
  SITE 1: note = The N-terminus is modified by an acetyl group
  SITE 38: note = The C-terminus is modified by an amino group
  SITE 38: note = The C-terminal is modified by a cholesterol molecule
TYEEYEKKIEELEKKIEELLKKAEEQQKKNEQEAAAKK

SEQ ID NO: 16 - protein, 36 aa, synthetic construct
  SITE 1: note = The N-terminus is modified by an acetyl group
  SITE 36: note = The C-terminus is modified by an amino group
  SITE 36: note = The C-terminal is modified by a cholesterol molecule
TYEEYEKKIEELEKKIEELLKKAEEQQKKNEAAAKK

SEQ ID NO: 17 - protein, 36 aa, synthetic construct
  SITE 1: note = The N-terminus is modified by an acetyl group
  SITE 36: note = The C-terminus is modified by an amino group
  SITE 36: note = The C-terminal is modified by a cholesterol molecule
EYEEYEKKIEELEKKIEELLKKAEEQQKKNEAAAKK

SEQ ID NO: 18 - protein, 36 aa, synthetic construct
  SITE 1: note = The N-terminus is modified by an acetyl group
  SITE 36: note = The C-terminus is modified by an amino group
  SITE 36: note = The C-terminal is modified by a cholesterol molecule
EYEEYEKELEELEKKIEELLKKAEEQQKKNEAAAKK

SEQ ID NO: 19 - protein, 33 aa, synthetic construct
  SITE 1: note = The N-terminus is modified by an acetyl group
  SITE 33: note = The C-terminus is modified by an amino group
  SITE 33: note = The C-terminal is modified by a cholesterol molecule
EYEKELEELEKKIEELLKKAEEQQKKNEAAAKK

SEQ ID NO: 20 - protein, 44 aa, synthetic construct
  SITE 1: note = The N-terminus is modified by an acetyl group
  SITE 44: note = The C-terminus is modified by an amino group
TVQARQLLSGIVQQQNNLLRAIEAQQHLLQLTVWGIKQLQARIL

SEQ ID NO: 21 - protein, 40 aa, synthetic construct; identical to SEQ ID NO: 11
  SITE 1: note = The N-terminus is modified by an acetyl group
  SITE 40: note = The C-terminus is modified by an amino group

SEQ ID NO: 22 - protein, 38 aa, synthetic construct; identical to SEQ ID NO: 12
  SITE 1: note = The N-terminus is modified by an acetyl group
  SITE 38: note = The C-terminus is modified by an amino group

SEQ ID NO: 23 - protein, 38 aa, synthetic construct; identical to SEQ ID NO: 13
  SITE 1: note = The N-terminus is modified by an acetyl group
  SITE 38: note = The C-terminus is modified by an amino group

SEQ ID NO: 24 - protein, 36 aa, synthetic construct; identical to SEQ ID NO: 14
  SITE 1: note = The N-terminus is modified by an acetyl group
  SITE 36: note = The C-terminus is modified by an amino group

SEQ ID NO: 25 - protein, 38 aa, synthetic construct; identical to SEQ ID NO: 15
  SITE 1: note = The N-terminus is modified by an acetyl group
  SITE 38: note = The C-terminus is modified by an amino group

SEQ ID NO: 26 - protein, 36 aa, synthetic construct; identical to SEQ ID NO: 16
  SITE 1: note = The N-terminus is modified by an acetyl group
  SITE 36: note = The C-terminus is modified by an amino group

SEQ ID NO: 27 - protein, 36 aa, synthetic construct; identical to SEQ ID NO: 17
  SITE 1: note = The N-terminus is modified by an acetyl group
  SITE 36: note = The C-terminus is modified by an amino group

SEQ ID NO: 28 - protein, 36 aa, synthetic construct; identical to SEQ ID NO: 18
  SITE 1: note = The N-terminus is modified by an acetyl group
  SITE 36: note = The C-terminus is modified by an amino group

SEQ ID NO: 29 - protein, 33 aa, synthetic construct; identical to SEQ ID NO: 19
  SITE 1: note = The N-terminus is modified by an acetyl group
  SITE 33: note = The C-terminus is modified by an amino group